European Patent Specification EP 3 924 008 B1, published April 9, 2025. Title: VASCULARIZING DEVICES AND METHODS FOR IMPLANTED DIAGNOSTICS AND THERAPEUTICS. Applicant: WILLIAM MARSH RICE UNIVERSITY. Application Unknown. The sequence listing filed with the application follows.

SEQUENCE LISTING (2 sequences)

SEQ ID NO: 1 - protein, 12 aa, Artificial sequence
  Synthetic peptide
CGPQGIWGQGCR

SEQ ID NO: 2 - protein, 6 aa, Artificial sequence
  Synthetic peptide
CGRGDS